European Patent Application EP 4 703 481 A1, published March 4, 2026. Title: METHOD FOR DETECTING MYCOBACTERIUM SPECIES IN FISH. Applicant: TSIAMIS GEORGIOS. Application EP. The sequence listing filed with the application follows.

SEQUENCE LISTING (9 sequences)

SEQ ID NO: 1 - DNA, 19 bp, synthetic construct
  source 1..19: mol_type = other DNA
aatccgaggtctccttcgc

SEQ ID NO: 2 - DNA, 20 bp, synthetic construct
  source 1..20: mol_type = other DNA
gtcggtggtgatgtcgaacc

SEQ ID NO: 3 - DNA, 18 bp, synthetic construct
  source 1..18: mol_type = other DNA
gcggtcgacggtgaggtc

SEQ ID NO: 4 - DNA, 20 bp, synthetic construct
  source 1..20: mol_type = other DNA
ggctctgctccagctcactt

SEQ ID NO: 5 - DNA, 269 bp, synthetic construct
  source 1..269: mol_type = other DNA
aatccgaggtctccttcgccacctacttcaatgcgtttccggccagctactggcgacgctggtcgatctgtaagtccgtggtgctgcgcgtcgagttgtccggtgccgggcgcgtcgacgtctaccggaccaaggccaccggagcgcgcatcttcgtcgaagggcgcgcatttgccggtgatgaggacaagccggccgtgctcgagatcgaggtggcgctgacgccgtttgaagacggcggctggatctggttcgacatcaccaccgac

SEQ ID NO: 6 - DNA, 380 bp, synthetic construct
  source 1..380: mol_type = other DNA
aatccgaggtctccttcgcgacctacttcaacgccttcccggccagttactggcgccgctggtcgacgctggaatcagtggtgttgcgtgtcgaactcaccggcagcgcgcgcgtcgacgtctaccggtccaaggccaccgggtcccggataaccgtcggcggggcgccgatctccagcgaaaatgtcggcgcgagcgcctcgggatctgatggcggcgcaagcgcctcgggatctgatgtcggcgcaagcgcctcgggatctgatgtcggcgcaagcgcctcgggatctgatgtcggcgcgagcgcctccgtggagttcgaggtcgacctcaccccgttcgaggacggtggctggatctggttcgacatcaccaccgac

SEQ ID NO: 7 - DNA, 538 bp, synthetic construct
  source 1..538: mol_type = other DNA
gcggtcgagggtgaggtcgaagtggccgctgaggccgaagaggctgaggcgggcgaggacgagccaaaagaggcagaagaggtcgctgaggccgaggggtctgaggccgaggacaagacagcgcaggccatagatggtggccaaaagggggttgacgaggcaggcgaggccgatgctgagccagacgacgactccaccgcggcagaacccgaggtcgtggtcgagcaagcagatatcgaagagatcgaaccccaagagcccgaagcggaggcggtggcggccgctgaagcgacggacgccgacgagggtgatggcgagcccgccgagccggcgagcgacgatctcgacgctgtcgcggccgaggacgctgacgttgacgttgacgccacggcaaccgaagccgaagaatccggcgatgagtcgcccgagcccgccgcagactccgaggagcccgaagccgacgagtccgcaccggaggactcggccgaggacacttcgtccggtgaatccgacacccaaagtgagttggagcagagcc

SEQ ID NO: 8 - DNA, 831 bp, synthetic construct
  source 1..831: mol_type = other DNA
catgggaccccaccacgcttcgttgtcgcggtaccaggtgatggtgtcgcgcaggccggcctcgaagtcggtgtgcgccggcttccagcccagctcgtcacgcagcggtgacggatcgatcgcgtaccgcagatcgtggcccacccggtcggtgacgtggtcgaactcgtcggtgggtcggtccatcagcgtcaggatcgtgcgcatcacggacagattgtcgtgttcgccgtcggctccgatcagatacgtgcgcccgatctcgccgtctgcgaggatccgccacaccgcactgttgtggtcgtcgacatggatccagtcgcgcacattggcaccgctgccgtacagcttggggcgccggccggtcagcacattggtgatctggcgcggaatgaacttctcgacatgctggtaggggccgtagttgttggagcagttcgagatcgtcgccgccaccccgtaggagcgcacccacgcccggaccagcatgtcggccgccgccttggtcgacgagtacgggctggacgggttgtacgcagtcgactcggtgaatcgtcgcggatcgtcgagcgtcagatcgccgtacacctcgtcggtggacacatggtgcaaccggatgcccgcctcagaacctctgtggcgcaccgcttccagtaccgagaacgtaccgaggacattcgaccgcacgaacggctcgggatcggccagtgcgttgtcgacgtgggtctccgcggcgaagtgcaccaccgcatcggactcggcgacgagcttgcccaccagcggcgcatcggtgatatcaccctgcaccaaccggatctcaccgtcgaccgc

SEQ ID NO: 9 - DNA, 904 bp, synthetic construct
  source 1..904: mol_type = other DNA
gcggtcgacggtgaggtcgaggcggctgaggcgggcgaggtagaggttgctgaggcggtcgagggtgaggttgaggcggctgaggcgggcgaggtagaggttgctgaggcggtcgagggtgaggttgaggcggctgctgaggctgagatgcctgagctgggtgaggtagaagctgctgaggaggccgatgaggcgggngagggngaggtagaagcggttgaggaggcggctgaggccgaggcacccgaggtgggtgaggtagaggttgctgaggcggtcgacggtgaggttgaggaggcggctgagcctgaagaggctgaggttgaggaggcggctgagcctgaagaggctgaggcgggngaggnagaggttgctgaggcgatcgagggnggggtcgacgaggccgctgaggccgaagaggctgaggcgggcgaggacgagccaaaagaggcagcagaggtcgctgaggccgaggggtctgaggccgaggacaagacagcgcaggccatagatggtggccaaacgggggttgacgacgcagacgaggccgatgctgagccagacgacgactccaccgcggcagaacccgaggtcgtggtcgagcaagcagatatcgaagagatcgaaccccaagagcccgaagcggaggcattggcggccgctgaagcgacggacgccgacgagggtgatggcgagcccgccgagccggcgagcgacgatctcgacgctgtcgcggccgaggacgctgacgccacggcaaccgaagccgaagaatccggcgatgagtcgcccgagcccgccgcagactccgaggagcccggagccgacgagtccgcaccggaggactcagccgaggacacttcgtccggtgaatccgacacccaaagtgagctggagcagagcc